European Patent Application EP 4 574 132 A1, published June 25, 2025. Title: Magnetic Torquer Conjugate-Based Drug. Applicant: UIF (University Industry Foundation), Yonsei University. The sequence listing filed with the application follows.

SEQUENCE LISTING (2 sequences)

SEQ ID NO: 1 - protein, 762 aa, synthetic construct
MGSYLHEPPGDEPSMRIEQPKTADRAPEQVAIHICEPSKVVTESFPFSETAEPEAKSKNCPCPEIARIGPCPNKPPKIPINRGLSRISTNKSRPKSRFGEPSWPVESSLDLTSQSPVSPYREEAFSVENCGTAGSRRGSFARGTTSRAASSSRKDETKEGPDEKEVYQRVTAQLSARNQKRMTVKLMIELSVFLCLLGCLVCSLTVDGFKRYTVIGLDIWKWFLLLLVIFSGMLITHWIVHVAVFFVEWKFLMRKNVLYFTHGLKTSVEVFIWITVVLATWVMLIKPDVNQPHEQKLISEEDLQTRKILEFVTWTIVTVLIGAFLWLVKTTLLKILASSFHLNRFFDRIQESVFHHSVLQTLAGRPVVELAQGISRTESQDGAGQVSFMEHTKTQNKKVVDVGKLHQMKQEKVPAWTMQLLVDVVSNSGLSTMSGMLDEDMVEGGVELDDDEITNEEQAIATAVRIFDNIVQDKVDQSYIDRVDLHRFLIWEEVDHLFPLFEVNEKGQISLKAFAKWVVKVYNDQAALKHALNDNKTAVKQLNKLVTAILIVMMIVIWLIVTGIATTKLIVLLSSQLVVAAFIFGNTCKTIFEAIIFVFVMHPFDVGDRCVIDGNKMLVEEMNILTTVFLKWDKEKVYYPNSILCTKAIGNFFRSPDQGDVLEFSVDFTTPVLKIGDLKDRIKMYLEQNLNFWHPQHNMVVKEIENVNKIKMALFVNHTINFQDFAEKNRRRSELVLELKKIFEELDIKYNLLPQEISIRNM

SEQ ID NO: 2 - protein, 10 aa, synthetic construct
EQKLISEEDL